European Patent Specification EP 3 781 708 B1, published January 15, 2025. Title: METHOD AND APPARATUS FOR DETECTING A PLURALITY OF TARGET NUCLEIC ACID SEQUENCES IN SAMPLE. Applicant: SEEGENE, INC. The sequence listing filed with the application follows.

SEQUENCE LISTING (12 sequences)

SEQ ID NO: 1 - DNA, 35 bp, Artificial Sequence
  Synthetic nucleotide: 33-F
  misc_feature (22)..(26): n is deoxyinosine
aatggtatttgttggggcaatnnnnnatttgttac

SEQ ID NO: 2 - DNA, 37 bp, Artificial Sequence
  Synthetic nucleotide: 33-R
  misc_feature (6): n is deoxyinosine
  misc_feature (13): s is guanine or cytosine
  misc_feature (24)..(28): n is deoxyinosine
tcctgnaaactascagatggaggnnnnnttaaaccaa

SEQ ID NO: 3 - DNA, 49 bp, Artificial Sequence
  Synthetic nucleotide: 33-PTO
  misc_feature (20): r is adenine or guanine
aacggtacgacggcacacargtaactagtgacagtacatataaaaatga

SEQ ID NO: 4 - DNA, 38 bp, Artificial Sequence
  Synthetic nucleotide: 33-CTO
ttatattttattttattatatactgccgtcgtaccgtt

SEQ ID NO: 5 - DNA, 40 bp, Artificial Sequence
  Synthetic nucleotide: 39-F
  misc_feature (3): y is cytosine or thymine
  misc_feature (27)..(31): n is deoxyinosine
gayactacccgtagtaccaactttacnnnnnctacctcta

SEQ ID NO: 6 - DNA, 33 bp, Artificial Sequence
  Synthetic nucleotide: 39-R
  misc_feature (20)..(24): n is deoxyinosine
  misc_feature (27): r is adenine or guanine
ctggcagatggtggaggagnnnnngcraaattc

SEQ ID NO: 7 - DNA, 42 bp, Artificial Sequence
  Synthetic nucleotide: 39-PTO
  misc_feature (28): k is guanine or thymine
  misc_feature (29): r is adenine or guanine
acggcgcaatacctcctccacgtgcctkrtatattccttaaa

SEQ ID NO: 8 - DNA, 38 bp, Artificial Sequence
  Synthetic nucleotide: 39-CTO
tattattattaagagctgcttccgaggtattgcgccgt

SEQ ID NO: 9 - DNA, 33 bp, Artificial Sequence
  Synthetic nucleotide: 52-F
  misc_feature (20)..(24): n is deoxyinosine
cagggccacaataatggcannnnntggggcaat

SEQ ID NO: 10 - DNA, 34 bp, Artificial Sequence
  Synthetic nucleotide: 52-R
  misc_feature (22)..(26): n is deoxyinosine
  misc_feature (32): w is adenine or thymine
cctttcctttaggtggtgtgtnnnnntgacawgt

SEQ ID NO: 11 - DNA, 44 bp, Artificial Sequence
  Synthetic nucleotide: 52-PTO
  misc_feature (40): y is cytosine or thymine
tgtcgatcgcgtccagtcctctaaaatagtggcatccatyttat

SEQ ID NO: 12 - DNA, 38 bp, Artificial Sequence
  Synthetic nucleotide: 52-CTO
tgcgatatgtcgggtacgactggtggacgcgatcgaca